European Patent Application EP 4 365 590 A2, published May 8, 2024. Title: AGENT TARGETING DOUBLE-MEMBRANE ORGANELLE DNA. Applicant: Juntendo Educational Foundation. The sequence listing filed with the application follows.

SEQUENCE LISTING (30 sequences)

SEQ ID NO: 1 - DNA, 21 bp, synthetic construct
  misc_feature 1..21: note = Primer
  source 1..21: mol_type = other DNA
acacattcgaagaacccgtat

SEQ ID NO: 2 - DNA, 21 bp, synthetic construct
  misc_feature 1..21: note = Primer
  source 1..21: mol_type = other DNA
tttagttggggcatttcactg

SEQ ID NO: 3 - DNA, 30 bp, synthetic construct
  misc_feature 1..30: note = Primer
  source 1..30: mol_type = other DNA
tgacggggtcacccacactgtgcccatcta

SEQ ID NO: 4 - DNA, 30 bp, synthetic construct
  misc_feature 1..30: note = Primer
  source 1..30: mol_type = other DNA
ctagaagcatttgcggtggacgatggaggg

SEQ ID NO: 5 - DNA, 22 bp, synthetic construct
  misc_feature 1..22: note = Primer
  source 1..22: mol_type = other DNA
ttcacaaagcgccttcccccgt

SEQ ID NO: 6 - DNA, 23 bp, synthetic construct
  misc_feature 1..23: note = Primer
  source 1..23: mol_type = other DNA
gcgatggtgagagctaaggtcgg

SEQ ID NO: 7 - DNA, 20 bp, synthetic construct
  misc_feature 1..20: note = Primer
  source 1..20: mol_type = other DNA
ctgacgagatcatgaagaca

SEQ ID NO: 8 - DNA, 20 bp, synthetic construct
  misc_feature 1..20: note = Primer
  source 1..20: mol_type = other DNA
agtttgctggcaaagtagaa

SEQ ID NO: 9 - DNA, 24 bp, synthetic construct
  misc_feature 1..24: note = Primer
  source 1..24: mol_type = other DNA
gcactcagaggaggcgccatgtca

SEQ ID NO: 10 - DNA, 22 bp, synthetic construct
  misc_feature 1..22: note = Primer
  source 1..22: mol_type = other DNA
ggacgagacgacgtcccctgtc

SEQ ID NO: 11 - DNA, 24 bp, synthetic construct
  misc_feature 1..24: note = Primer
  source 1..24: mol_type = other DNA
gcttgcttgttacacacacaggtc

SEQ ID NO: 12 - DNA, 24 bp, synthetic construct
  misc_feature 1..24: note = Primer
  source 1..24: mol_type = other DNA
gcagaacaatcagcaatttcaagg

SEQ ID NO: 13 - DNA, 20 bp, synthetic construct
  misc_feature 1..20: note = Primer
  source 1..20: mol_type = other DNA
cgaccactttgtcaagctca

SEQ ID NO: 14 - DNA, 20 bp, synthetic construct
  misc_feature 1..20: note = Primer
  source 1..20: mol_type = other DNA
aggggtctacatggcaagtg

SEQ ID NO: 15 - DNA, 20 bp, synthetic construct
  misc_feature 1..20: note = Primer
  source 1..20: mol_type = other DNA
cattggcgtttgagtcagca

SEQ ID NO: 16 - DNA, 20 bp, synthetic construct
  misc_feature 1..20: note = Primer
  source 1..20: mol_type = other DNA
catggagtgggccatagctt

SEQ ID NO: 17 - DNA, 20 bp, synthetic construct
  misc_feature 1..20: note = Primer
  source 1..20: mol_type = other DNA
cagaagtacctgagctcgcc

SEQ ID NO: 18 - DNA, 20 bp, synthetic construct
  misc_feature 1..20: note = Primer
  source 1..20: mol_type = other DNA
agattcgtagctggatgccg

SEQ ID NO: 19 - DNA, 20 bp, synthetic construct
  misc_feature 1..20: note = Primer
  source 1..20: mol_type = other DNA
gttgtgcaagggtctggttt

SEQ ID NO: 20 - DNA, 20 bp, synthetic construct
  misc_feature 1..20: note = Primer
  source 1..20: mol_type = other DNA
ggatggtgtctcttgcagga

SEQ ID NO: 21 - DNA, 20 bp, synthetic construct
  misc_feature 1..20: note = Primer
  source 1..20: mol_type = other DNA
atgacttccaagctggccgt

SEQ ID NO: 22 - DNA, 20 bp, synthetic construct
  misc_feature 1..20: note = Primer
  source 1..20: mol_type = other DNA
tccttggcaaaactgcacct

SEQ ID NO: 23 - DNA, 20 bp, synthetic construct
  misc_feature 1..20: note = Primer
  source 1..20: mol_type = other DNA
cggtaccggcgggcattcag

SEQ ID NO: 24 - DNA, 20 bp, synthetic construct
  misc_feature 1..20: note = Primer
  source 1..20: mol_type = other DNA
cggctctcggctgctgcatt

SEQ ID NO: 25 - DNA, 20 bp, synthetic construct
  misc_feature 1..20: note = Primer
  source 1..20: mol_type = other DNA
ctgagcagatcatgaagaca

SEQ ID NO: 26 - DNA, 20 bp, synthetic construct
  misc_feature 1..20: note = Primer
  source 1..20: mol_type = other DNA
agtttgctggcaaagtagaa

SEQ ID NO: 27 - DNA, 20 bp, synthetic construct
  misc_feature 1..20: note = Primer
  source 1..20: mol_type = other DNA
ctttgagttcggtggggtca

SEQ ID NO: 28 - DNA, 20 bp, synthetic construct
  misc_feature 1..20: note = Primer
  source 1..20: mol_type = other DNA
gggccgtacagttccacaaa

SEQ ID NO: 29 - DNA, 20 bp, synthetic construct
  misc_feature 1..20: note = Primer
  source 1..20: mol_type = other DNA
ggaccaccgcatctctacat

SEQ ID NO: 30 - DNA, 20 bp, synthetic construct
  misc_feature 1..20: note = Primer
  source 1..20: mol_type = other DNA
gttcctctatggggtcgtca